European Patent Specification EP 4 291 664 B1, published May 27, 2026. Title: SITE-SPECIFIC GENOME MODIFICATION TECHNOLOGY. Applicant: NORTH CAROLINA STATE UNIVERSITY. The sequence listing filed with the application follows.

SEQUENCE LISTING (38 sequences)

SEQ ID NO: 1 - protein, 1624 aa, Artificial sequence
  Synthetic
MAYDYSASLNPQKALIWRIVHRDNIPWILDNGLHCGNSLVQAENWINIDNPELIGKRAGHPVPVGTGGTLHDYVPFYFTPFSPMLMNIHSGRGGIKRRPNEEIVILVSNLRNVAAHDVPFVFTDSHAYYNWTNYYTSLNSLDQIDWPILQARDFRRDPDDPAKFERYQAEALIWQHCPISLLDGIICYSEEVRLQLEQWLFQRNLTMSVHTRSGWYFSSGGSSGGSSGSETPGTSESATPESSGGSSGGSEKKYSIGLAIGTNSVGWAVITDDYKVPSKKFKVLGNTNRKSIKKNLMGALLFDSGETAEATRLKRTARRRYTRRKNRIRYLQEIFANEMAKLDDSFFQRLEESFLVEEDKKNERHPIFGNLADEVAYHRNYPTIYHLRKKLADSPEKADLRLIYLALAHIIKFRGHFLIEGKLNAENSDVAKLFYQLIQTYNQLFEESPLDEIEVDAKGILSARLSKSKRLEKLIAVFPNEKKNGLFGNIIALALGLTPNFKSNFDLTEDAKLQLSKDTYDDDLDELLGQIGDQYADLFSAAKNLSDAILLSDILRSNSEVTKAPLSASMVKRYDEHHQDLALLKTLVRQQFPEKYAEIFKDDTKNGYAGYVGIGIKHRKRTTKLATQEEFYKFIKPILEKMDGAEELLAKLNRDDLLRKQRTFDNGSIPHQIHLKELHAILRRQEEFYPFLKENREKIEKILTFRIPYYVGPLARGNSRFAWLTRKSEEAITPWNFEEVVDKGASAQSFIERMTNFDEQLPNKKVLPKHSLLYEYFTVYNELTKVKYVTERMRKPEFLSGEQKKAIVDLLFKTNRKVTVKQLKEDYFKKIECFDSVEIIGVEDRFNASLGTYHDLLKIIKDKDFLDNEENEDILEDIVLTLTLFEDREMIEERLKTYAHLFDDKVMKQLKRRHYTGWGRLSRKMINGIRDKQSGKTILDFLKSDGFSNRNFMQLIHDDSLTFKEEIEKAQVSGQGDSLHEQIADLAGSPAIKKGILQTVKIVDELVKVMGHKPENIVIEMARENQTTTKGLQQSRERKKRIEEGIKELESQILKENPVENTQLQNEKLYLYYLQNGRDMYVDQELDINRLSDYDVDAIVPQSFIKDDSIDNKVLTRSVENRGKSDNVPSEEVVKKMKNYWRQLLNAKLITQRKFDNLTKAERGGLSEADKAGFIKRQLVETRQITKHVARILDSRMNTKRDKNDKPIREVKVITLKSKLVSDFRKDFQLYKVRDINNYHHAHDAYLNAVVGTALIKKYPKLESEFVYGDYKVYDVRKMIAKSEQEIGKATAKRFFYSNIMNFFKTEVKLANGEIRKRPLIETNGETGEVVWNKEKDFATVRKVLAMPQVNIVKKTEVQTGGFSKESILSKRESAKLIPRKKGWDTRKYGGFGSPTVAYSILVVAKVEKGKAKKLKSVKVLVGITIMEKGSYEKDPIGFLEAKGYKDIKKELIFKLPKYSLFELENGRRRMLASATELQKANELVLPQHLVRLLYYTQNISATTGSNNLGYIEQHREEFKEIFEKIIDFSEKYILKNKVNSNLKSSFDEQFAVSDSILLSNSFVSLLKYTSFGASGGFTFLDLDVKQGRLRYQTVTEVLDATLIYQSITGLYETRTDLSQLGGD

SEQ ID NO: 2 - protein, 1624 aa, Artificial sequence
  Synthetic
MAYDYSASLNPQKALIWRIVHRDNIPWILDNGLHCGNSLVQAENWINIDNPELIGARAGHPVPVGTGGTLHDYVPFYFTPFSPMLMNIHSGRGGIKRRPNEEIVILVSNLRNVAAHDVPFVFTDSHAYYNWTNYYTSLNSLDQIDWPILQARDFRRDPDDPAKFERYQAEALIWQHCPISLLDGIICYSEEVRLQLEQWLFQRNLTMSVHTRSGWYFSSGGSSGGSSGSETPGTSESATPESSGGSSGGSEKKYSIGLAIGTNSVGWAVITDDYKVPSKKFKVLGNTNRKSIKKNLMGALLFDSGETAEATRLKRTARRRYTRRKNRIRYLQEIFANEMAKLDDSFFQRLEESFLVEEDKKNERHPIFGNLADEVAYHRNYPTIYHLRKKLADSPEKADLRLIYLALAHIIKFRGHFLIEGKLNAENSDVAKLFYQLIQTYNQLFEESPLDEIEVDAKGILSARLSKSKRLEKLIAVFPNEKKNGLFGNIIALALGLTPNFKSNFDLTEDAKLQLSKDTYDDDLDELLGQIGDQYADLFSAAKNLSDAILLSDILRSNSEVTKAPLSASMVKRYDEHHQDLALLKTLVRQQFPEKYAEIFKDDTKNGYAGYVGIGIKHRKRTTKLATQEEFYKFIKPILEKMDGAEELLAKLNRDDLLRKQRTFDNGSIPHQIHLKELHAILRRQEEFYPFLKENREKIEKILTFRIPYYVGPLARGNSRFAWLTRKSEEAITPWNFEEVVDKGASAQSFIERMTNFDEQLPNKKVLPKHSLLYEYFTVYNELTKVKYVTERMRKPEFLSGEQKKAIVDLLFKTNRKVTVKQLKEDYFKKIECFDSVEIIGVEDRFNASLGTYHDLLKIIKDKDFLDNEENEDILEDIVLTLTLFEDREMIEERLKTYAHLFDDKVMKQLKRRHYTGWGRLSRKMINGIRDKQSGKTILDFLKSDGFSNRNFMQLIHDDSLTFKEEIEKAQVSGQGDSLHEQIADLAGSPAIKKGILQTVKIVDELVKVMGHKPENIVIEMARENQTTTKGLQQSRERKKRIEEGIKELESQILKENPVENTQLQNEKLYLYYLQNGRDMYVDQELDINRLSDYDVDAIVPQSFIKDDSIDNKVLTRSVENRGKSDNVPSEEVVKKMKNYWRQLLNAKLITQRKFDNLTKAERGGLSEADKAGFIKRQLVETRQITKHVARILDSRMNTKRDKNDKPIREVKVITLKSKLVSDFRKDFQLYKVRDINNYHHAHDAYLNAVVGTALIKKYPKLESEFVYGDYKVYDVRKMIAKSEQEIGKATAKRFFYSNIMNFFKTEVKLANGEIRKRPLIETNGETGEVVWNKEKDFATVRKVLAMPQVNIVKKTEVQTGGFSKESILSKRESAKLIPRKKGWDTRKYGGFGSPTVAYSILVVAKVEKGKAKKLKSVKVLVGITIMEKGSYEKDPIGFLEAKGYKDIKKELIFKLPKYSLFELENGRRRMLASATELQKANELVLPQHLVRLLYYTQNISATTGSNNLGYIEQHREEFKEIFEKIIDFSEKYILKNKVNSNLKSSFDEQFAVSDSILLSNSFVSLLKYTSFGASGGFTFLDLDVKQGRLRYQTVTEVLDATLIYQSITGLYETRTDLSQLGGD

SEQ ID NO: 3 - protein, 1624 aa, Artificial sequence
  Synthetic
MAYDYSASLNPQKALIWRIVHRDNIPWILDNGLHCGNSLVQAENWINIDNPELIGKRAGHPVPVGTGGTLHDYVPFYFTPFSPMLMNIHSGRGGIKRRPNEEIVILVSNLRNVAAHDVPFVFTDSHAYYNWTNYYTSLNSLDQIDWPILQARDFRRDPDDPAKFERYQAEALIWQHCPISLLDGIICYSEEVRLQLEQWLFQRNLTMSVHTRSGWYFSSGGSSGGSSGSETPGTSESATPESSGGSSGGSEKKYSIGLAIGTNSVGWAVITDDYKVPSKKFKVLGNTNRKSIKKNLMGALLFDSGETAEATRLKRTARRRYTRRKNRIRYLQEIFANEMAKLDDSFFQRLEESFLVEEDKKNERHPIFGNLADEVAYHRNYPTIYHLRKKLADSPEKADLRLIYLALAHIIKFRGHFLIEGKLNAENSDVAKLFYQLIQTYNQLFEESPLDEIEVDAKGILSARLSKSKRLEKLIAVFPNEKKNGLFGNIIALALGLTPNFKSNFDLTEDAKLQLSKDTYDDDLDELLGQIGDQYADLFSAAKNLSDAILLSDILRSNSEVTKAPLSASMVKRYDEHHQDLALLKTLVRQQFPEKYAEIFKDDTKNGYAGYVGIGIKHRKRTTKLATQEEFYKFIKPILEKMDGAEELLAKLNRDDLLRKQRTFDNGSIPHQIHLKELHAILRRQEEFYPFLKENREKIEKILTFRIPYYVGPLARGNSRFAWLTRKSEEAITPWNFEEVVDKGASAQSFIERMTNFDEQLPNKKVLPKHSLLYEYFTVYNELTKVKYVTERMRKPEFLSGEQKKAIVDLLFKTNRKVTVKQLKEDYFKKIECFDSVEIIGVEDRFNASLGTYHDLLKIIKDKDFLDNEENEDILEDIVLTLTLFEDREMIEERLKTYAHLFDDKVMKQLKRRHYTGWGRLSRKMINGIRDKQSGKTILDFLKSDGFSNRNFMQLIHDDSLTFKEEIEKAQVSGQGDSLHEQIADLAGSPAIKKGILQTVKIVDELVKVMGHKPENIVIEMARENQTTTKGLQQSRERKKRIEEGIKELESQILKENPVENTQLQNEKLYLYYLQNGRDMYVDQELDINRLSDYDVDHIVPQSFIKDDSIDNKVLTRSVENRGKSDNVPSEEVVKKMKNYWRQLLNAKLITQRKFDNLTKAERGGLSEADKAGFIKRQLVETRQITKHVARILDSRMNTKRDKNDKPIREVKVITLKSKLVSDFRKDFQLYKVRDINNYHHAHDAYLNAVVGTALIKKYPKLESEFVYGDYKVYDVRKMIAKSEQEIGKATAKRFFYSNIMNFFKTEVKLANGEIRKRPLIETNGETGEVVWNKEKDFATVRKVLAMPQVNIVKKTEVQTGGFSKESILSKRESAKLIPRKKGWDTRKYGGFGSPTVAYSILVVAKVEKGKAKKLKSVKVLVGITIMEKGSYEKDPIGFLEAKGYKDIKKELIFKLPKYSLFELENGRRRMLASATELQKANELVLPQHLVRLLYYTQNISATTGSNNLGYIEQHREEFKEIFEKIIDFSEKYILKNKVNSNLKSSFDEQFAVSDSILLSNSFVSLLKYTSFGASGGFTFLDLDVKQGRLRYQTVTEVLDATLIYQSITGLYETRTDLSQLGGD

SEQ ID NO: 4 - protein, 1624 aa, Artificial sequence
  Synthetic
MAYDYSASLNPQKALIWRIVHRDNIPWILDNGLHCGNSLVQAENWINIDNPELIGARAGHPVPVGTGGTLHDYVPFYFTPFSPMLMNIHSGRGGIKRRPNEEIVILVSNLRNVAAHDVPFVFTDSHAYYNWTNYYTSLNSLDQIDWPILQARDFRRDPDDPAKFERYQAEALIWQHCPISLLDGIICYSEEVRLQLEQWLFQRNLTMSVHTRSGWYFSSGGSSGGSSGSETPGTSESATPESSGGSSGGSEKKYSIGLAIGTNSVGWAVITDDYKVPSKKFKVLGNTNRKSIKKNLMGALLFDSGETAEATRLKRTARRRYTRRKNRIRYLQEIFANEMAKLDDSFFQRLEESFLVEEDKKNERHPIFGNLADEVAYHRNYPTIYHLRKKLADSPEKADLRLIYLALAHIIKFRGHFLIEGKLNAENSDVAKLFYQLIQTYNQLFEESPLDEIEVDAKGILSARLSKSKRLEKLIAVFPNEKKNGLFGNIIALALGLTPNFKSNFDLTEDAKLQLSKDTYDDDLDELLGQIGDQYADLFSAAKNLSDAILLSDILRSNSEVTKAPLSASMVKRYDEHHQDLALLKTLVRQQFPEKYAEIFKDDTKNGYAGYVGIGIKHRKRTTKLATQEEFYKFIKPILEKMDGAEELLAKLNRDDLLRKQRTFDNGSIPHQIHLKELHAILRRQEEFYPFLKENREKIEKILTFRIPYYVGPLARGNSRFAWLTRKSEEAITPWNFEEVVDKGASAQSFIERMTNFDEQLPNKKVLPKHSLLYEYFTVYNELTKVKYVTERMRKPEFLSGEQKKAIVDLLFKTNRKVTVKQLKEDYFKKIECFDSVEIIGVEDRFNASLGTYHDLLKIIKDKDFLDNEENEDILEDIVLTLTLFEDREMIEERLKTYAHLFDDKVMKQLKRRHYTGWGRLSRKMINGIRDKQSGKTILDFLKSDGFSNRNFMQLIHDDSLTFKEEIEKAQVSGQGDSLHEQIADLAGSPAIKKGILQTVKIVDELVKVMGHKPENIVIEMARENQTTTKGLQQSRERKKRIEEGIKELESQILKENPVENTQLQNEKLYLYYLQNGRDMYVDQELDINRLSDYDVDHIVPQSFIKDDSIDNKVLTRSVENRGKSDNVPSEEVVKKMKNYWRQLLNAKLITQRKFDNLTKAERGGLSEADKAGFIKRQLVETRQITKHVARILDSRMNTKRDKNDKPIREVKVITLKSKLVSDFRKDFQLYKVRDINNYHHAHDAYLNAVVGTALIKKYPKLESEFVYGDYKVYDVRKMIAKSEQEIGKATAKRFFYSNIMNFFKTEVKLANGEIRKRPLIETNGETGEVVWNKEKDFATVRKVLAMPQVNIVKKTEVQTGGFSKESILSKRESAKLIPRKKGWDTRKYGGFGSPTVAYSILVVAKVEKGKAKKLKSVKVLVGITIMEKGSYEKDPIGFLEAKGYKDIKKELIFKLPKYSLFELENGRRRMLASATELQKANELVLPQHLVRLLYYTQNISATTGSNNLGYIEQHREEFKEIFEKIIDFSEKYILKNKVNSNLKSSFDEQFAVSDSILLSNSFVSLLKYTSFGASGGFTFLDLDVKQGRLRYQTVTEVLDATLIYQSITGLYETRTDLSQLGGD

SEQ ID NO: 5 - protein, 355 aa, Artificial sequence
  Synthetic
MITYTQGNLLDAPVEALVNTVNTVGVMGKGIALMFKERFPENMKVYALACKQKQVITGKMFITETGELMGPRWIVNFPTKQHWRADSRMEWIEDGLQDLRRFLIEENVQSIAIPPLGAGNGGLNWPDVRAQIESALGDLQDVDILIYQPTEKYQNVAKSTGVKKLTPARAAIAELVRRYWVLGMECSLLEIQKLAWLLQRAIEQHQQDDILKLRFEAHYYGPYAPNLNHLLNALDGTYLKAEKRIPDSQPLDVIWFNDQKKEHVNAYLNNEAREWLPALEQVSQLIDGFESPFGLELLATVDWLLSRGECQPTLDSVKEGLHQWPAGERWASRKLRLFDNNNLQFAINRVMEFHC

SEQ ID NO: 6 - protein, 230 aa, Artificial sequence
  Synthetic
MDVRAQIESALGDLQDVDILIYQPTEKYQNVAKSTGVKKLTPARAAIAELVRRYWVLGMECSLLEIQKLAWLLQRAIEQHQQDDILKLRFEAHYYGPYAPNLNHLLNALDGTYLKAEKRIPDSQPLDVIWFNDQKKEHVNAYLNNEAREWLPALEQVSQLIDGFESPFGLELLATVDWLLSRGECQPTLDSVKEGLHQWPAGERWASRKLRLFDNNNLQFAINRVMEFHC

SEQ ID NO: 7 - protein, 126 aa, Artificial sequence
  Synthetic
MITYTQGNLLDAPVEALVNTVNTVGVMGKGIALMFKERFPENMKVYALACKQKQVITGKMFITETGELMGPRWIVNFPTKQHWRADSRMEWIEDGLQDLRRFLIEENVQSIAIPPLGAGNGGLNWP

SEQ ID NO: 8 - protein, 241 aa, Artificial sequence
  Synthetic
MPASIPRRNIVGKEKKSRILTKPCVIEYEGQIVGYGSKELRVETISCWLARTIIQTKHYSRRFVNNSYLHLGVFSGRDLVGVLQWGYALNPNSGRRVVLETDNRGYMELNRMWLHDDMPRNSESRAISYALKVIRLLYPSVEWVQSFADERCGRAGVVYQASNFDFIGSHESTFYELDGEWYHEITMNAIKRGGQRGVYLRANKERAVVHKFNQYRYIRFLNKRARKRLNTKLFKVQPYPK

SEQ ID NO: 9 - protein, 241 aa, Artificial sequence
  Synthetic
MPASIPRRNIVGKEKKSRILTKPCVIEYEGQIVGYGSKELRVETISCWLARTIIQTKHYSRRFVNNSYLHLGVFSGRDLVGVLQWGYALNPNSGRRVVLETDNRGYMELNRMWLHDDMPRNSESRAISYALKVIRLLYPSVEWVQSFAAERCGRAGVVYQASNFDFIGSHESTFYELDGEWYHEITMNAIKRGGQRGVYLRANKERAVVHKFNQYRYIRFLNKRARKRLNTKLFKVQPYPK

SEQ ID NO: 10 - protein, 1647 aa, Artificial sequence
  Synthetic
MPASIPRRNIVGKEKKSRILTKPCVIEYEGQIVGYGSKELRVETISCWLARTIIQTKHYSRRFVNNSYLHLGVFSGRDLVGVLQWGYALNPNSGRRVVLETDNRGYMELNRMWLHDDMPRNSESRAISYALKVIRLLYPSVEWVQSFAAERCGRAGVVYQASNFDFIGSHESTFYELDGEWYHEITMNAIKRGGQRGVYLRANKERAVVHKFNQYRYIRFLNKRARKRLNTKLFKVQPYPKSGGSSGGSSGSETPGTSESATPESSGGSSGGSEKKYSIGLAIGTNSVGWAVITDDYKVPSKKFKVLGNTNRKSIKKNLMGALLFDSGETAEATRLKRTARRRYTRRKNRIRYLQEIFANEMAKLDDSFFQRLEESFLVEEDKKNERHPIFGNLADEVAYHRNYPTIYHLRKKLADSPEKADLRLIYLALAHIIKFRGHFLIEGKLNAENSDVAKLFYQLIQTYNQLFEESPLDEIEVDAKGILSARLSKSKRLEKLIAVFPNEKKNGLFGNIIALALGLTPNFKSNFDLTEDAKLQLSKDTYDDDLDELLGQIGDQYADLFSAAKNLSDAILLSDILRSNSEVTKAPLSASMVKRYDEHHQDLALLKTLVRQQFPEKYAEIFKDDTKNGYAGYVGIGIKHRKRTTKLATQEEFYKFIKPILEKMDGAEELLAKLNRDDLLRKQRTFDNGSIPHQIHLKELHAILRRQEEFYPFLKENREKIEKILTFRIPYYVGPLARGNSRFAWLTRKSEEAITPWNFEEVVDKGASAQSFIERMTNFDEQLPNKKVLPKHSLLYEYFTVYNELTKVKYVTERMRKPEFLSGEQKKAIVDLLFKTNRKVTVKQLKEDYFKKIECFDSVEIIGVEDRFNASLGTYHDLLKIIKDKDFLDNEENEDILEDIVLTLTLFEDREMIEERLKTYAHLFDDKVMKQLKRRHYTGWGRLSRKMINGIRDKQSGKTILDFLKSDGFSNRNFMQLIHDDSLTFKEEIEKAQVSGQGDSLHEQIADLAGSPAIKKGILQTVKIVDELVKVMGHKPENIVIEMARENQTTTKGLQQSRERKKRIEEGIKELESQILKENPVENTQLQNEKLYLYYLQNGRDMYVDQELDINRLSDYDVDAIVPQSFIKDDSIDNKVLTRSVENRGKSDNVPSEEVVKKMKNYWRQLLNAKLITQRKFDNLTKAERGGLSEADKAGFIKRQLVETRQITKHVARILDSRMNTKRDKNDKPIREVKVITLKSKLVSDFRKDFQLYKVRDINNYHHAHDAYLNAVVGTALIKKYPKLESEFVYGDYKVYDVRKMIAKSEQEIGKATAKRFFYSNIMNFFKTEVKLANGEIRKRPLIETNGETGEVVWNKEKDFATVRKVLAMPQVNIVKKTEVQTGGFSKESILSKRESAKLIPRKKGWDTRKYGGFGSPTVAYSILVVAKVEKGKAKKLKSVKVLVGITIMEKGSYEKDPIGFLEAKGYKDIKKELIFKLPKYSLFELENGRRRMLASATELQKANELVLPQHLVRLLYYTQNISATTGSNNLGYIEQHREEFKEIFEKIIDFSEKYILKNKVNSNLKSSFDEQFAVSDSILLSNSFVSLLKYTSFGASGGFTFLDLDVKQGRLRYQTVTEVLDATLIYQSITGLYETRTDLSQLGGD

SEQ ID NO: 11 - protein, 200 aa, Artificial sequence
  Synthetic
MRRRAAAVVLSLSAVLATSAATAPAQTPTATATSAKAAAPACPRFDDPVHAAADPRVDVERITPDPVWRTTCGTLYRSDSRGPAVVFEQGFLPKDVIDGQYDIESYVLVNQPSPYVSTTYDHDLYKTWYKSGYNYYIDAPGGVDVNKTIGDRHKWADQVEVAFPGGIRTEFVIGVCPVDKKTRTEKMSECVGNPHYEPWH

SEQ ID NO: 12 - protein, 200 aa, Artificial sequence
  Synthetic
MRRRAAAVVLSLSAVLATSAATAPAQTPTATATSAKAAAPACPRFDDPVHAAADPRVDVERITPDPVWRTTCGTLYRSDSRGPAVVFEQGFLPKDVIDGQYDIESYVLVNQPSPYVSTTYDHDLYKTWYASGYNYYIDAPGGVDVNKTIGDRHKWADQVEVAFPGGIRTEFVIGVCPVDKKTRTEKMSECVGNPHYEPWH

SEQ ID NO: 13 - protein, 1806 aa, Artificial sequence
  Synthetic
MRRRAAAVVLSLSAVLATSAATAPAQTPTATATSAKAAAPACPRFDDPVHAAADPRVDVERITPDPVWRTTCGTLYRSDSRGPAVVFEQGFLPKDVIDGQYDIESYVLVNQPSPYVSTTYDHDLYKTWYASGYNYYIDAPGGVDVNKTIGDRHKWADQVEVAFPGGIRTEFVIGVCPVDKKTRTEKMSECVGNPHYEPWHMRRRAAAVVLSLSAVLATSAATAPAQTPTATATSAKAAAPACPRFDDPVHAAADPRVDVERITPDPVWRTTCGTLYRSDSRGPAVVFEQGFLPKDVIDGQYDIESYVLVNQPSPYVSTTYDHDLYKTWYASGYNYYIDAPGGVDVNKTIGDRHKWADQVEVAFPGGIRTEFVIGVCPVDKKTRTEKMSECVGNPHYEPWHSGGSSGGSSGSETPGTSESATPESSGGSSGGSEKKYSIGLAIGTNSVGWAVITDDYKVPSKKFKVLGNTNRKSIKKNLMGALLFDSGETAEATRLKRTARRRYTRRKNRIRYLQEIFANEMAKLDDSFFQRLEESFLVEEDKKNERHPIFGNLADEVAYHRNYPTIYHLRKKLADSPEKADLRLIYLALAHIIKFRGHFLIEGKLNAENSDVAKLFYQLIQTYNQLFEESPLDEIEVDAKGILSARLSKSKRLEKLIAVFPNEKKNGLFGNIIALALGLTPNFKSNFDLTEDAKLQLSKDTYDDDLDELLGQIGDQYADLFSAAKNLSDAILLSDILRSNSEVTKAPLSASMVKRYDEHHQDLALLKTLVRQQFPEKYAEIFKDDTKNGYAGYVGIGIKHRKRTTKLATQEEFYKFIKPILEKMDGAEELLAKLNRDDLLRKQRTFDNGSIPHQIHLKELHAILRRQEEFYPFLKENREKIEKILTFRIPYYVGPLARGNSRFAWLTRKSEEAITPWNFEEVVDKGASAQSFIERMTNFDEQLPNKKVLPKHSLLYEYFTVYNELTKVKYVTERMRKPEFLSGEQKKAIVDLLFKTNRKVTVKQLKEDYFKKIECFDSVEIIGVEDRFNASLGTYHDLLKIIKDKDFLDNEENEDILEDIVLTLTLFEDREMIEERLKTYAHLFDDKVMKQLKRRHYTGWGRLSRKMINGIRDKQSGKTILDFLKSDGFSNRNFMQLIHDDSLTFKEEIEKAQVSGQGDSLHEQIADLAGSPAIKKGILQTVKIVDELVKVMGHKPENIVIEMARENQTTTKGLQQSRERKKRIEEGIKELESQILKENPVENTQLQNEKLYLYYLQNGRDMYVDQELDINRLSDYDVDAIVPQSFIKDDSIDNKVLTRSVENRGKSDNVPSEEVVKKMKNYWRQLLNAKLITQRKFDNLTKAERGGLSEADKAGFIKRQLVETRQITKHVARILDSRMNTKRDKNDKPIREVKVITLKSKLVSDFRKDFQLYKVRDINNYHHAHDAYLNAVVGTALIKKYPKLESEFVYGDYKVYDVRKMIAKSEQEIGKATAKRFFYSNIMNFFKTEVKLANGEIRKRPLIETNGETGEVVWNKEKDFATVRKVLAMPQVNIVKKTEVQTGGFSKESILSKRESAKLIPRKKGWDTRKYGGFGSPTVAYSILVVAKVEKGKAKKLKSVKVLVGITIMEKGSYEKDPIGFLEAKGYKDIKKELIFKLPKYSLFELENGRRRMLASATELQKANELVLPQHLVRLLYYTQNISATTGSNNLGYIEQHREEFKEIFEKIIDFSEKYILKNKVNSNLKSSFDEQFAVSDSILLSNSFVSLLKYTSFGASGGFTFLDLDVKQGRLRYQTVTEVLDATLIYQSITGLYETRTDLSQLGGD

SEQ ID NO: 14 - protein, 218 aa, Artificial sequence
  Synthetic
MAYDYSASLNPQKALIWRIVHRDNIPWILDNGLHCGNSLVQAENWINIDNPELIGKRAGHPVPVGTGGTLHDYVPFYFTPFSPMLMNIHSGRGGIKRRPNEEIVILVSNLRNVAAHDVPFVFTDSHAYYNWTNYYTSLNSLDQIDWPILQARDFRRDPDDPAKFERYQAEALIWQHCPISLLDGIICYSEEVALQLEQWLFQRNLTMSVHTRSGWYFS

SEQ ID NO: 15 - protein, 1624 aa, Artificial sequence
  Synthetic
MAYDYSASLNPQKALIWRIVHRDNIPWILDNGLHCGNSLVQAENWINIDNPELIGKRAGHPVPVGTGGTLHDYVPFYFTPFSPMLMNIHSGRGGIKRRPNEEIVILVSNLRNVAAHDVPFVFTDSHAYYNWTNYYTSLNSLDQIDWPILQARDFRRDPDDPAKFERYQAEALIWQHCPISLLDGIICYSEEVALQLEQWLFQRNLTMSVHTRSGWYFSSGGSSGGSSGSETPGTSESATPESSGGSSGGSEKKYSIGLAIGTNSVGWAVITDDYKVPSKKFKVLGNTNRKSIKKNLMGALLFDSGETAEATRLKRTARRRYTRRKNRIRYLQEIFANEMAKLDDSFFQRLEESFLVEEDKKNERHPIFGNLADEVAYHRNYPTIYHLRKKLADSPEKADLRLIYLALAHIIKFRGHFLIEGKLNAENSDVAKLFYQLIQTYNQLFEESPLDEIEVDAKGILSARLSKSKRLEKLIAVFPNEKKNGLFGNIIALALGLTPNFKSNFDLTEDAKLQLSKDTYDDDLDELLGQIGDQYADLFSAAKNLSDAILLSDILRSNSEVTKAPLSASMVKRYDEHHQDLALLKTLVRQQFPEKYAEIFKDDTKNGYAGYVGIGIKHRKRTTKLATQEEFYKFIKPILEKMDGAEELLAKLNRDDLLRKQRTFDNGSIPHQIHLKELHAILRRQEEFYPFLKENREKIEKILTFRIPYYVGPLARGNSRFAWLTRKSEEAITPWNFEEVVDKGASAQSFIERMTNFDEQLPNKKVLPKHSLLYEYFTVYNELTKVKYVTERMRKPEFLSGEQKKAIVDLLFKTNRKVTVKQLKEDYFKKIECFDSVEIIGVEDRFNASLGTYHDLLKIIKDKDFLDNEENEDILEDIVLTLTLFEDREMIEERLKTYAHLFDDKVMKQLKRRHYTGWGRLSRKMINGIRDKQSGKTILDFLKSDGFSNRNFMQLIHDDSLTFKEEIEKAQVSGQGDSLHEQIADLAGSPAIKKGILQTVKIVDELVKVMGHKPENIVIEMARENQTTTKGLQQSRERKKRIEEGIKELESQILKENPVENTQLQNEKLYLYYLQNGRDMYVDQELDINRLSDYDVDAIVPQSFIKDDSIDNKVLTRSVENRGKSDNVPSEEVVKKMKNYWRQLLNAKLITQRKFDNLTKAERGGLSEADKAGFIKRQLVETRQITKHVARILDSRMNTKRDKNDKPIREVKVITLKSKLVSDFRKDFQLYKVRDINNYHHAHDAYLNAVVGTALIKKYPKLESEFVYGDYKVYDVRKMIAKSEQEIGKATAKRFFYSNIMNFFKTEVKLANGEIRKRPLIETNGETGEVVWNKEKDFATVRKVLAMPQVNIVKKTEVQTGGFSKESILSKRESAKLIPRKKGWDTRKYGGFGSPTVAYSILVVAKVEKGKAKKLKSVKVLVGITIMEKGSYEKDPIGFLEAKGYKDIKKELIFKLPKYSLFELENGRRRMLASATELQKANELVLPQHLVRLLYYTQNISATTGSNNLGYIEQHREEFKEIFEKIIDFSEKYILKNKVNSNLKSSFDEQFAVSDSILLSNSFVSLLKYTSFGASGGFTFLDLDVKQGRLRYQTVTEVLDATLIYQSITGLYETRTDLSQLGGD

SEQ ID NO: 16 - protein, 218 aa, Artificial sequence
  Synthetic
MAYDYSASLNPQKALIWRIVHRDNIPWILDNGLHCGNSLVQAENWINIDNPELIGKRAGHPVPVGTGGTLHDYVPFYFTPFSPMLLNIHSGAGGIKRRPNEEIVILVSNLRNVAAHDVPFVFTDSHAYYNWTNYYTSLNSLDQIDWPILQARDFRRDPDDPAKFERYQAEALIWQHCPISLLDGIICYSEEVALQLEQWLFQRNLTMSVHTRSGWYFS

SEQ ID NO: 17 - protein, 1624 aa, Artificial sequence
  Synthetic
MAYDYSASLNPQKALIWRIVHRDNIPWILDNGLHCGNSLVQAENWINIDNPELIGKRAGHPVPVGTGGTLHDYVPFYFTPFSPMLLNIHSGAGGIKRRPNEEIVILVSNLRNVAAHDVPFVFTDSHAYYNWTNYYTSLNSLDQIDWPILQARDFRRDPDDPAKFERYQAEALIWQHCPISLLDGIICYSEEVALQLEQWLFQRNLTMSVHTRSGWYFSSGGSSGGSSGSETPGTSESATPESSGGSSGGSEKKYSIGLAIGTNSVGWAVITDDYKVPSKKFKVLGNTNRKSIKKNLMGALLFDSGETAEATRLKRTARRRYTRRKNRIRYLQEIFANEMAKLDDSFFQRLEESFLVEEDKKNERHPIFGNLADEVAYHRNYPTIYHLRKKLADSPEKADLRLIYLALAHIIKFRGHFLIEGKLNAENSDVAKLFYQLIQTYNQLFEESPLDEIEVDAKGILSARLSKSKRLEKLIAVFPNEKKNGLFGNIIALALGLTPNFKSNFDLTEDAKLQLSKDTYDDDLDELLGQIGDQYADLFSAAKNLSDAILLSDILRSNSEVTKAPLSASMVKRYDEHHQDLALLKTLVRQQFPEKYAEIFKDDTKNGYAGYVGIGIKHRKRTTKLATQEEFYKFIKPILEKMDGAEELLAKLNRDDLLRKQRTFDNGSIPHQIHLKELHAILRRQEEFYPFLKENREKIEKILTFRIPYYVGPLARGNSRFAWLTRKSEEAITPWNFEEVVDKGASAQSFIERMTNFDEQLPNKKVLPKHSLLYEYFTVYNELTKVKYVTERMRKPEFLSGEQKKAIVDLLFKTNRKVTVKQLKEDYFKKIECFDSVEIIGVEDRFNASLGTYHDLLKIIKDKDFLDNEENEDILEDIVLTLTLFEDREMIEERLKTYAHLFDDKVMKQLKRRHYTGWGRLSRKMINGIRDKQSGKTILDFLKSDGFSNRNFMQLIHDDSLTFKEEIEKAQVSGQGDSLHEQIADLAGSPAIKKGILQTVKIVDELVKVMGHKPENIVIEMARENQTTTKGLQQSRERKKRIEEGIKELESQILKENPVENTQLQNEKLYLYYLQNGRDMYVDQELDINRLSDYDVDAIVPQSFIKDDSIDNKVLTRSVENRGKSDNVPSEEVVKKMKNYWRQLLNAKLITQRKFDNLTKAERGGLSEADKAGFIKRQLVETRQITKHVARILDSRMNTKRDKNDKPIREVKVITLKSKLVSDFRKDFQLYKVRDINNYHHAHDAYLNAVVGTALIKKYPKLESEFVYGDYKVYDVRKMIAKSEQEIGKATAKRFFYSNIMNFFKTEVKLANGEIRKRPLIETNGETGEVVWNKEKDFATVRKVLAMPQVNIVKKTEVQTGGFSKESILSKRESAKLIPRKKGWDTRKYGGFGSPTVAYSILVVAKVEKGKAKKLKSVKVLVGITIMEKGSYEKDPIGFLEAKGYKDIKKELIFKLPKYSLFELENGRRRMLASATELQKANELVLPQHLVRLLYYTQNISATTGSNNLGYIEQHREEFKEIFEKIIDFSEKYILKNKVNSNLKSSFDEQFAVSDSILLSNSFVSLLKYTSFGASGGFTFLDLDVKQGRLRYQTVTEVLDATLIYQSITGLYETRTDLSQLGGD

SEQ ID NO: 18 - protein, 5 aa, Artificial sequence
  Synthetic
  misc_feature (1)..(1): Xaa can be L, I, V, or A
  misc_feature (2)..(2): Xaa can be I, Q, K, T, or N
  misc_feature (3)..(4): Xaa can be any naturally occurring amino acid
XXXXR

SEQ ID NO: 19 - protein, 21 aa, Artificial sequence
  Synthetic
  misc_feature (1)..(4): Xaa can be any naturally occurring amino acid
  misc_feature (5)..(5): Xaa can be L, V, or I
  misc_feature (6)..(6): Xaa can be H, G, N, S, or A
  misc_feature (7)..(7): Xaa can be D or E
  misc_feature (8)..(8): Xaa can be Y or F
  misc_feature (9)..(9): Xaa can be V, I, or A
  misc_feature (14)..(14): Xaa can be T, A, G, K, N, or W
  misc_feature (15)..(16): Xaa can be any naturally occurring amino acid
  misc_feature (17)..(17): Xaa can be S, T, N, M, or K
  misc_feature (18)..(18): Xaa can be P, V, M, I, A
  misc_feature (20)..(20): Xaa can be L, M or F
  misc_feature (21)..(21): Xaa can be any naturally occurring amino acid
XXXXXXXXXPFYFXXXXXMXX

SEQ ID NO: 20 - protein, 8 aa, Artificial sequence
  Synthetic
  misc_feature (1)..(1): Xaa can be F, Y, W, V, or C
  misc_feature (2)..(2): Xaa can be V, L, I, A, C, or F
  misc_feature (3)..(3): Xaa can be F, Y, or A
  misc_feature (4)..(4): Xaa can be T, S, Y, or F
  misc_feature (5)..(5): Xaa can be D, N, or S
  misc_feature (6)..(6): Xaa can be G, R, S, A, M or Q
  misc_feature (7)..(7): Xaa can be H, N, S, or Q
  misc_feature (8)..(8): Xaa can be A, G, C, H or K
XXXXXXXX

SEQ ID NO: 21 - protein, 9 aa, Artificial sequence
  Synthetic
  misc_feature (1)..(1): Xaa can be any naturally occurring amino acid
  misc_feature (2)..(2): Xaa can be R, K, H, E, F, L, T, or M
  misc_feature (3)..(3): Xaa can be Y, R, K, D, E, or H
  misc_feature (4)..(4): Xaa can be Q, M, E, Y, A, R, or H;
  misc_feature (5)..(5): Xaa can be A Q, S, or Y
  misc_feature (6)..(6): Xaa can be E, A, or Q
  misc_feature (7)..(7): Xaa can be F, A, L, E, V, or C
  misc_feature (8)..(8): Xaa can be L, A, E, or M
  misc_feature (9)..(9): Xaa can be V, I, L, or A
XXXXXXXXX

SEQ ID NO: 22 - protein, 14 aa, Artificial sequence
  Synthetic
  misc_feature (1)..(4): Xaa can be any naturally occurring amino acid
  misc_feature (5)..(5): Xaa can be Q, E, or R
  misc_feature (6)..(6): Xaa can be any naturally occurring amino acid
  misc_feature (8)..(8): Xaa can be V or I
  misc_feature (9)..(9): Xaa can be A, L, V, S, or T
  misc_feature (10)..(10): Xaa can be F, I, V, or L
  misc_feature (11)..(11): Xaa can be P, A, or I
  misc_feature (14)..(14): Xaa can be I, V, or L
XXXXXXEXXXXGGX

SEQ ID NO: 23 - protein, 7 aa, Artificial sequence
  Synthetic
  misc_feature (1)..(1): Xaa can be S, T, or G
  misc_feature (2)..(2): Xaa can be any naturally occurring amino acid
  misc_feature (3)..(3): Xaa can be F, Y, or L
  misc_feature (4)..(4): Xaa can be V, I, A, or L
  misc_feature (5)..(5): Xaa can be S, G, or A
  misc_feature (6)..(6): Xaa can be T or A
  misc_feature (7)..(7): Xaa can be T, S, or A
XXXXXXX

SEQ ID NO: 24 - protein, 7 aa, Artificial sequence
  Synthetic
  misc_feature (1)..(1): Xaa can be L or V
  misc_feature (2)..(2): Xaa can be any naturally occurring amino acid
  misc_feature (3)..(3): Xaa can be R, H, or K
  misc_feature (4)..(4): Xaa can be any naturally occurring amino acid
  misc_feature (5)..(5): Xaa can be D, S, or A
  misc_feature (6)..(6): Xaa can be any naturally occurring amino acid
  misc_feature (7)..(7): Xaa can be R or D
XXXXXXX

SEQ ID NO: 25 - protein, 5 aa, Artificial sequence
  Synthetic
  misc_feature (1)..(1): Xaa can be any naturally occurring amino acid
  misc_feature (4)..(4): Xaa can be S or L
  misc_feature (5)..(5): Xaa can be H, G, K, R, N, D, or A
XHYXX

SEQ ID NO: 26 - protein, 17 aa, Artificial sequence
  Synthetic
  misc_feature (2)..(2): Xaa can be L, I, or F
  misc_feature (3)..(3): Xaa can be N, G, S, or T
  misc_feature (4)..(4): Xaa can be R or K
  misc_feature (5)..(5): Xaa can be M, L, or A
  misc_feature (6)..(6): Xaa can be W, A, C, V, F, or Y
  misc_feature (7)..(7): Xaa can be L, I, F, M, V, C, or T
  misc_feature (8)..(8): Xaa can be any naturally occurring amino acid
  misc_feature (9)..(9): Xaa can be D or E
  misc_feature (10)..(10): Xaa can be any naturally occurring amino acid
  misc_feature (11)..(11): Xaa can be L ,A, M, C, V, Q, or T
  misc_feature (12)..(12): Xaa can be P, G, A, or L
  misc_feature (13)..(13): Xaa can be R, K, H, T, or M
  misc_feature (14)..(14): Xaa can be N or F
  misc_feature (15)..(15): Xaa can be S, A, T, or G
  misc_feature (17)..(17): Xaa can be S or T
EXXXXXXXXXXXXXXEX

SEQ ID NO: 27 - protein, 18 aa, Artificial sequence
  Synthetic
  misc_feature (1)..(1): Xaa can be F, W, Y, or M
  misc_feature (2)..(2): Xaa can be A or S
  misc_feature (4)..(4): Xaa can be E, G, P, A, or T
  misc_feature (5)..(6): Xaa can be any naturally occurring amino acid
  misc_feature (7)..(7): Xaa can be G, C, or Q
  misc_feature (8)..(9): Xaa can be any naturally occurring amino acid
  misc_feature (11)..(11): Xaa can be T, V, Y, or I
  misc_feature (12)..(12): Xaa can be V or I
  misc_feature (14)..(14): Xaa can be Q, K, or R
  misc_feature (16)..(16): Xaa can be A, S, C, T, or N
  misc_feature (17)..(17): Xaa can be N, G, or A
  misc_feature (18)..(18): Xaa can be F, W, or Y
XXDXXXXXXGXXYXAXXX

SEQ ID NO: 28 - DNA, 37 bp, Artificial sequence
  Synthetic
tggaaaactgtgggtagtaggagggcaaagtgtacaa

SEQ ID NO: 29 - DNA, 49 bp, Artificial sequence
  Synthetic
caaaagtaagggcgagaaatattgatagtaaagaggtcacgaggttgtt

SEQ ID NO: 30 - DNA, 27 bp, Artificial sequence
  Synthetic
tttccgttgataaacgttgctgcataa

SEQ ID NO: 31 - DNA, 27 bp, Artificial sequence
  Synthetic
tttaatgaatgaaacagccgcgctgta

SEQ ID NO: 32 - DNA, 27 bp, Artificial sequence
  Synthetic
ccggctgtgccgtgagccaccatcaaa

SEQ ID NO: 33 - DNA, 27 bp, Artificial sequence
  Synthetic
tttgccgtaatagtaagacctgagcgc

SEQ ID NO: 34 - DNA, 27 bp, Artificial sequence
  Synthetic
cgttgctgcattgataatctacacaaa

SEQ ID NO: 35 - DNA, 27 bp, Artificial sequence
  Synthetic
ttccggcacgttgatcggtgccggaaa

SEQ ID NO: 36 - DNA, 27 bp, Artificial sequence
  Synthetic
gtctcaattcatgggtcaaaataaccc

SEQ ID NO: 37 - DNA, 27 bp, Artificial sequence
  Synthetic
gtctcaattcatgggtcaaaacaaccc

SEQ ID NO: 38 - DNA, 27 bp, Artificial sequence
  Synthetic
gtctcaattcatgggtcaaaataaccc